European Patent Application EP 4 520 350 A1, published March 12, 2025. Title: Fusion protein comprising GLP-1, immunoglobulin Fc, and IGF-1 and Use thereof. Applicant: ImmunoForge Co.,Ltd. The sequence listing filed with the application follows.

SEQUENCE LISTING (42 sequences)

SEQ ID NO: 1 - protein, 36 aa, Homo sapiens
HDEFERHAEGTFTSDVSSYLEGQAAKEFIAWLVKGR

SEQ ID NO: 2 - protein, 30 aa, Homo sapiens
HAEGTFTSDVSSYLEGQAAKEFIAWLVKGR

SEQ ID NO: 3 - protein, 31 aa, Homo sapiens
HGEGTFTSDVSSYLEEQAAKEFIAWLVKGGG

SEQ ID NO: 4 - protein, 227 aa, synthetic construct
DKTHTCPPCPAPELLGGPSVFLFPPKPKDTLMISRTPEVTCVVVDVSHEDPEVKFNWYVDGVEVHNAKTKPREEQYNSTYRVVSVLTVLHQDWLNGKEYKCKVSNKALPAPIEKTISKAKGQPREPQVYTLPPSREEMTKNQVSLTCLVKGFYPSDIAVEWESNGQPENNYKTTPPVLDSDGSFFLYSKLTVDKSRWQQGNVFSCSVMHEALHNHYTQKSLSLSPGK

SEQ ID NO: 5 - protein, 227 aa, synthetic construct
DKTHTCPPCPAPELLGGPSVFLFPPKPKDTLMISRTPEVTCVVVDVSHEDPEVKFNWYVDGVEVHNAKTKPREEQYASTYRVVSVLTVLHQDWLNGKEYKCKVSNKALPAPIEKTISKAKGQPREPQVYTLPPSREEMTKNQVSLTCLVKGFYPSDIAVEWESNGQPENNYKTTPPVLDSDGSFFLYSKLTVDKSRWQQGNVFSCSVMHEALHNHYTQKSLSLSPGK

SEQ ID NO: 6 - protein, 227 aa, synthetic construct
DKTHTCPPCPAPELLGGPSVFLFPPKPKDTLMISRTPEVTCVVVDVSHEDPEVKFNWYVDGVEVHNAKTKPREEQYNSTYRVVSVLTVYHMDWLNGKEYKCKVSNKALPAPIEKTISKAKGQPREPQVYTLPPSREEMTKNQVSLTCLVKGFYPSDIAVEWESNGQPENNYKTTPPVLDSDGSFFLYSKLTVDKSRWQQGNVFSCSVLHEALHNHYTQKSLSLSPGK

SEQ ID NO: 7 - protein, 227 aa, synthetic construct
DKTHTCPPCPAPELLGGPSVFLFPPKPKDTLMISRTPEVTCVVVDVSHEDPEVKFNWYVDGVEVHNAKTKPREEQYNSTYRVVSVLTVEHMDWLNGKEYKCKVSNKALPAPIEKTISKAKGQPREPQVYTLPPSREEMTKNQVSLTCLVKGFYPSDIAVEWESNGQPENNYKTTPPVLDSDGSFFLYSKLTVDKSRWQQGNVFSCSVLHEALHNHYTQKSLSLSPGK

SEQ ID NO: 8 - protein, 227 aa, synthetic construct
DKTHTCPPCPAPELLGGPSVFLFPPKPKDTLMISRTPEVTCVVVDVSHEDPEVKFNWYVDGVEVHNAKTKPREEQYNSTYRVVSVLTVEHWDWLNGKEYKCKVSNKALPAPIEKTISKAKGQPREPQVYTLPPSREEMTKNQVSLTCLVKGFYPSDIAVEWESNGQPENNYKTTPPVLDSDGSFFLYSKLTVDKSRWQQGNVFSCSVLHEALHNHYTQKSLSLSPGK

SEQ ID NO: 9 - protein, 70 aa, Homo sapiens
GPETLCGAELVDALQFVCGDRGFYFNKPTGYGSSSRRAPQTGIVDECCFRSCDLRRLEMYCAPLKPAKSA

SEQ ID NO: 10 - protein, 70 aa, synthetic construct
GPATLCGAELVDALQFVCGDRGFYFNKPTGYGSSSRRAPQTGIVDECCARSCDLRRLEMYCAPLKPAKSA

SEQ ID NO: 11 - protein, 70 aa, synthetic construct
GPETLCGAELVDALQFVCGDRGFYFNKPTGYGSSSRRAPQTGIVDECCFRSCDLRRLEMYCAPLKPTKST

SEQ ID NO: 12 - protein, 70 aa, synthetic construct
GPATLCGAELVDALQFVCGDRGFYFNKPTGYGSSSRRAPQTGIVDECCARSCDLRRLEMYCAPLKPTKST

SEQ ID NO: 13 - protein, 363 aa, synthetic construct
HGEGTFTSDVSSYLEEQAAKEFIAWLVKGGGGSAPAPGGGGSDKTHTCPPCPAPELLGGPSVFLFPPKPKDTLMISRTPEVTCVVVDVSHEDPEVKFNWYVDGVEVHNAKTKPREEQYNSTYRVVSVLTVLHQDWLNGKEYKCKVSNKALPAPIEKTISKAKGQPREPQVYTLPPSREEMTKNQVSLTCLVKGFYPSDIAVEWESNGQPENNYKTTPPVLDSDGSFFLYSKLTVDKSRWQQGNVFSCSVMHEALHNHYTQKSLSLSPGKGGGGSGGGGSGGGGSGGGGSGAHSGPETLCGAELVDALQFVCGDRGFYFNKPTGYGSSSRRAPQTGIVDECCFRSCDLRRLEMYCAPLKPAKSA

SEQ ID NO: 14 - protein, 363 aa, synthetic construct
HGEGTFTSDVSSYLEEQAAKEFIAWLVKGGGGSAPAPGGGGSDKTHTCPPCPAPELLGGPSVFLFPPKPKDTLMISRTPEVTCVVVDVSHEDPEVKFNWYVDGVEVHNAKTKPREEQYNSTYRVVSVLTVLHQDWLNGKEYKCKVSNKALPAPIEKTISKAKGQPREPQVYTLPPSREEMTKNQVSLTCLVKGFYPSDIAVEWESNGQPENNYKTTPPVLDSDGSFFLYSKLTVDKSRWQQGNVFSCSVMHEALHNHYTQKSLSLSPGKGGGGSGGGGSGGGGSGGGGSGAHSGPETLCGAELVDALQFVCGDRGFYFNKPTGYGSSSRRAPQTGIVDECCFRSCDLRRLEMYCAPLKPTKST

SEQ ID NO: 15 - protein, 363 aa, synthetic construct
HGEGTFTSDVSSYLEEQAAKEFIAWLVKGGGGSAPAPGGGGSDKTHTCPPCPAPELLGGPSVFLFPPKPKDTLMISRTPEVTCVVVDVSHEDPEVKFNWYVDGVEVHNAKTKPREEQYASTYRVVSVLTVLHQDWLNGKEYKCKVSNKALPAPIEKTISKAKGQPREPQVYTLPPSREEMTKNQVSLTCLVKGFYPSDIAVEWESNGQPENNYKTTPPVLDSDGSFFLYSKLTVDKSRWQQGNVFSCSVMHEALHNHYTQKSLSLSPGKGGGGSGGGGSGGGGSGGGGSGAHSGPETLCGAELVDALQFVCGDRGFYFNKPTGYGSSSRRAPQTGIVDECCFRSCDLRRLEMYCAPLKPAKSA

SEQ ID NO: 16 - protein, 363 aa, synthetic construct
HGEGTFTSDVSSYLEEQAAKEFIAWLVKGGGGSAPAPGGGGSDKTHTCPPCPAPELLGGPSVFLFPPKPKDTLMISRTPEVTCVVVDVSHEDPEVKFNWYVDGVEVHNAKTKPREEQYASTYRVVSVLTVLHQDWLNGKEYKCKVSNKALPAPIEKTISKAKGQPREPQVYTLPPSREEMTKNQVSLTCLVKGFYPSDIAVEWESNGQPENNYKTTPPVLDSDGSFFLYSKLTVDKSRWQQGNVFSCSVMHEALHNHYTQKSLSLSPGKGGGGSGGGGSGGGGSGGGGSGAHSGPETLCGAELVDALQFVCGDRGFYFNKPTGYGSSSRRAPQTGIVDECCFRSCDLRRLEMYCAPLKPTKST

SEQ ID NO: 17 - protein, 363 aa, synthetic construct
HGEGTFTSDVSSYLEEQAAKEFIAWLVKGGGGSAPAPGGGGSDKTHTCPPCPAPELLGGPSVFLFPPKPKDTLMISRTPEVTCVVVDVSHEDPEVKFNWYVDGVEVHNAKTKPREEQYASTYRVVSVLTVLHQDWLNGKEYKCKVSNKALPAPIEKTISKAKGQPREPQVYTLPPSREEMTKNQVSLTCLVKGFYPSDIAVEWESNGQPENNYKTTPPVLDSDGSFFLYSKLTVDKSRWQQGNVFSCSVMHEALHNHYTQKSLSLSPGKGGGGSGGGGSGGGGSGGGGSGAHSGPATLCGAELVDALQFVCGDRGFYFNKPTGYGSSSRRAPQTGIVDECCARSCDLRRLEMYCAPLKPAKSA

SEQ ID NO: 18 - protein, 363 aa, synthetic construct
HGEGTFTSDVSSYLEEQAAKEFIAWLVKGGGGSAPAPGGGGSDKTHTCPPCPAPELLGGPSVFLFPPKPKDTLMISRTPEVTCVVVDVSHEDPEVKFNWYVDGVEVHNAKTKPREEQYASTYRVVSVLTVLHQDWLNGKEYKCKVSNKALPAPIEKTISKAKGQPREPQVYTLPPSREEMTKNQVSLTCLVKGFYPSDIAVEWESNGQPENNYKTTPPVLDSDGSFFLYSKLTVDKSRWQQGNVFSCSVMHEALHNHYTQKSLSLSPGKGGGGSGGGGSGGGGSGGGGSGAHSGPATLCGAELVDALQFVCGDRGFYFNKPTGYGSSSRRAPQTGIVDECCARSCDLRRLEMYCAPLKPTKST

SEQ ID NO: 19 - protein, 386 aa, synthetic construct
HGEGTFTSDVSSYLEEQAAKEFIAWLVKGGGGSAPAPGGGGSDKTHTCPPCPAPELLGGPSVFLFPPKPKDTLMISRTPEVTCVVVDVSHEDPEVKFNWYVDGVEVHNAKTKPREEQYASTYRVVSVLTVLHQDWLNGKEYKCKVSNKALPAPIEKTISKAKGQPREPQVYTLPPSREEMTKNQVSLTCLVKGFYPSDIAVEWESNGQPENNYKTTPPVLDSDGSFFLYSKLTVDKSRWQQGNVFSCSVMHEALHNHYTQKSLSLSPGKGGGGSGGGGSGGGGSGGGGSGAHSGPETLCGAELVDALQFVCGDRGFYFNKPTGYGSSSRRAPQTGIVDECCFRSCDLRRLEMYCAPLKPAKSAGSAPAPGGGGSTHRPPMWSPVWP

SEQ ID NO: 20 - protein, 386 aa, synthetic construct
HGEGTFTSDVSSYLEEQAAKEFIAWLVKGGGGSAPAPGGGGSDKTHTCPPCPAPELLGGPSVFLFPPKPKDTLMISRTPEVTCVVVDVSHEDPEVKFNWYVDGVEVHNAKTKPREEQYASTYRVVSVLTVLHQDWLNGKEYKCKVSNKALPAPIEKTISKAKGQPREPQVYTLPPSREEMTKNQVSLTCLVKGFYPSDIAVEWESNGQPENNYKTTPPVLDSDGSFFLYSKLTVDKSRWQQGNVFSCSVMHEALHNHYTQKSLSLSPGKGGGGSGGGGSGGGGSGGGGSGAHSGPATLCGAELVDALQFVCGDRGFYFNKPTGYGSSSRRAPQTGIVDECCARSCDLRRLEMYCAPLKPTKSTGSAPAPGGGGSTHRPPMWSPVWP

SEQ ID NO: 21 - protein, 269 aa, synthetic construct
HGEGTFTSDVSSYLEEQAAKEFIAWLVKGGGGSAPAPGGGGSDKTHTCPPCPAPELLGGPSVFLFPPKPKDTLMISRTPEVTCVVVDVSHEDPEVKFNWYVDGVEVHNAKTKPREEQYASTYRVVSVLTVLHQDWLNGKEYKCKVSNKALPAPIEKTISKAKGQPREPQVYTLPPSREEMTKNQVSLTCLVKGFYPSDIAVEWESNGQPENNYKTTPPVLDSDGSFFLYSKLTVDKSRWQQGNVFSCSVMHEALHNHYTQKSLSLSPGK

SEQ ID NO: 22 - protein, 322 aa, synthetic construct
DKTHTCPPCPAPELLGGPSVFLFPPKPKDTLMISRTPEVTCVVVDVSHEDPEVKFNWYVDGVEVHNAKTKPREEQYASTYRVVSVLTVLHQDWLNGKEYKCKVSNKALPAPIEKTISKAKGQPREPQVYTLPPSREEMTKNQVSLTCLVKGFYPSDIAVEWESNGQPENNYKTTPPVLDSDGSFFLYSKLTVDKSRWQQGNVFSCSVMHEALHNHYTQKSLSLSPGKGGGGSGGGGSGGGGSGGGGSGAHSGPETLCGAELVDALQFVCGDRGFYFNKPTGYGSSSRRAPQTGIVDECCFRSCDLRRLEMYCAPLKPAKSAK

SEQ ID NO: 23 - protein, 321 aa, synthetic construct
DKTHTCPPCPAPELLGGPSVFLFPPKPKDTLMISRTPEVTCVVVDVSHEDPEVKFNWYVDGVEVHNAKTKPREEQYASTYRVVSVLTVLHQDWLNGKEYKCKVSNKALPAPIEKTISKAKGQPREPQVYTLPPSREEMTKNQVSLTCLVKGFYPSDIAVEWESNGQPENNYKTTPPVLDSDGSFFLYSKLTVDKSRWQQGNVFSCSVMHEALHNHYTQKSLSLSPGKGGGGSGGGGSGGGGSGGGGSGAHSGPATLCGAELVDALQFVCGDRGFYFNKPTGYGSSSRRAPQTGIVDECCARSCDLRRLEMYCAPLKPTKST

SEQ ID NO: 24 - protein, 344 aa, synthetic construct
DKTHTCPPCPAPELLGGPSVFLFPPKPKDTLMISRTPEVTCVVVDVSHEDPEVKFNWYVDGVEVHNAKTKPREEQYASTYRVVSVLTVLHQDWLNGKEYKCKVSNKALPAPIEKTISKAKGQPREPQVYTLPPSREEMTKNQVSLTCLVKGFYPSDIAVEWESNGQPENNYKTTPPVLDSDGSFFLYSKLTVDKSRWQQGNVFSCSVMHEALHNHYTQKSLSLSPGKGGGGSGGGGSGGGGSGGGGSGAHSGPATLCGAELVDALQFVCGDRGFYFNKPTGYGSSSRRAPQTGIVDECCARSCDLRRLEMYCAPLKPTKSTGSAPAPGGGGSTHRPPMWSPVWP

SEQ ID NO: 25 - protein, 363 aa, synthetic construct
HGEGTFTSDVSSYLEEQAAKEFIAWLVKGGGGSAPAPGGGGSDKTHTCPPCPAPELLGGPSVFLFPPKPKDTLMISRTPEVTCVVVDVSHEDPEVKFNWYVDGVEVHNAKTKPREEQYASTYRVVSVLTVYHMDWLNGKEYKCKVSNKALPAPIEKTISKAKGQPREPQVYTLPPSREEMTKNQVSLTCLVKGFYPSDIAVEWESNGQPENNYKTTPPVLDSDGSFFLYSKLTVDKSRWQQGNVFSCSVLHEALHNHYTQKSLSLSPGKGGGGSGGGGSGGGGSGGGGSGAHSGPATLCGAELVDALQFVCGDRGFYFNKPTGYGSSSRRAPQTGIVDECCARSCDLRRLEMYCAPLKPTKST

SEQ ID NO: 26 - protein, 363 aa, synthetic construct
HGEGTFTSDVSSYLEEQAAKEFIAWLVKGGGGSAPAPGGGGSDKTHTCPPCPAPELLGGPSVFLFPPKPKDTLMISRTPEVTCVVVDVSHEDPEVKFNWYVDGVEVHNAKTKPREEQYASTYRVVSVLTVEHMDWLNGKEYKCKVSNKALPAPIEKTISKAKGQPREPQVYTLPPSREEMTKNQVSLTCLVKGFYPSDIAVEWESNGQPENNYKTTPPVLDSDGSFFLYSKLTVDKSRWQQGNVFSCSVLHEALHNHYTQKSLSLSPGKGGGGSGGGGSGGGGSGGGGSGAHSGPATLCGAELVDALQFVCGDRGFYFNKPTGYGSSSRRAPQTGIVDECCARSCDLRRLEMYCAPLKPTKST

SEQ ID NO: 27 - protein, 363 aa, synthetic construct
HGEGTFTSDVSSYLEEQAAKEFIAWLVKGGGGSAPAPGGGGSDKTHTCPPCPAPELLGGPSVFLFPPKPKDTLMISRTPEVTCVVVDVSHEDPEVKFNWYVDGVEVHNAKTKPREEQYASTYRVVSVLTVEHWDWLNGKEYKCKVSNKALPAPIEKTISKAKGQPREPQVYTLPPSREEMTKNQVSLTCLVKGFYPSDIAVEWESNGQPENNYKTTPPVLDSDGSFFLYSKLTVDKSRWQQGNVFSCSVLHEALHNHYTQKSLSLSPGKGGGGSGGGGSGGGGSGGGGSGAHSGPATLCGAELVDALQFVCGDRGFYFNKPTGYGSSSRRAPQTGIVDECCARSCDLRRLEMYCAPLKPTKST

SEQ ID NO: 28 - protein, 354 aa, synthetic construct
HGEGTFTSDVSSYLEEQAAKEFIAWLVKGGGGSAPAPGGGGSDKTHTCPPCPAPELLGGPSVFLFPPKPKDTLMISRTPEVTCVVVDVSHEDPEVKFNWYVDGVEVHNAKTKPREEQYASTYRVVSVLTVLHQDWLNGKEYKCKVSNKALPAPIEKTISKAKGQPREPQVYTLPPSREEMTKNQVSLTCLVKGFYPSDIAVEWESNGQPENNYKTTPPVLDSDGSFFLYSKLTVDKSRWQQGNVFSCSVMHEALHNHYTQKSLSLSPGASGAGSTTLEVLFQGPGPATLCGAELVDALQFVCGDRGFYFNKPTGYGSSSRRAPQTGIVDECCARSCDLRRLEMYCAPLKPTKST

SEQ ID NO: 29 - protein, 346 aa, synthetic construct
HGEGTFTSDVSSYLEEQAAKEFIAWLVKGGGGSAPAPGGGGSDKTHTCPPCPAPELLGGPSVFLFPPKPKDTLMISRTPEVTCVVVDVSHEDPEVKFNWYVDGVEVHNAKTKPREEQYASTYRVVSVLTVLHQDWLNGKEYKCKVSNKALPAPIEKTISKAKGQPREPQVYTLPPSREEMTKNQVSLTCLVKGFYPSDIAVEWESNGQPENNYKTTPPVLDSDGSFFLYSKLTVDKSRWQQGNVFSCSVMHEALHNHYTQKSLSLSPGGGGGGGGGGPATLCGAELVDALQFVCGDRGFYFNKPTGYGSSSRRAPQTGIVDECCARSCDLRRLEMYCAPLKPTKST

SEQ ID NO: 30 - protein, 348 aa, synthetic construct
HGEGTFTSDVSSYLEEQAAKEFIAWLVKGGGGSAPAPGGGGSDKTHTCPPCPAPELLGGPSVFLFPPKPKDTLMISRTPEVTCVVVDVSHEDPEVKFNWYVDGVEVHNAKTKPREEQYASTYRVVSVLTVLHQDWLNGKEYKCKVSNKALPAPIEKTISKAKGQPREPQVYTLPPSREEMTKNQVSLTCLVKGFYPSDIAVEWESNGQPENNYKTTPPVLDSDGSFFLYSKLTVDKSRWQQGNVFSCSVMHEALHNHYTQKSLSLSPGPAPAPAPAPAGPATLCGAELVDALQFVCGDRGFYFNKPTGYGSSSRRAPQTGIVDECCARSCDLRRLEMYCAPLKPTKST

SEQ ID NO: 31 - protein, 268 aa, synthetic construct
HGEGTFTSDVSSYLEEQAAKEFIAWLVKGGGGSAPAPGGGGSDKTHTCPPCPAPELLGGPSVFLFPPKPKDTLMISRTPEVTCVVVDVSHEDPEVKFNWYVDGVEVHNAKTKPREEQYASTYRVVSVLTVLHQDWLNGKEYKCKVSNKALPAPIEKTISKAKGQPREPQVYTLPPSREEMTKNQVSLTCLVKGFYPSDIAVEWESNGQPENNYKTTPPVLDSDGSFFLYSKLTVDKSRWQQGNVFSCSVMHEALHNHYTQKSLSLSPG

SEQ ID NO: 32 - protein, 304 aa, synthetic construct
DKTHTCPPCPAPELLGGPSVFLFPPKPKDTLMISRTPEVTCVVVDVSHEDPEVKFNWYVDGVEVHNAKTKPREEQYASTYRVVSVLTVLHQDWLNGKEYKCKVSNKALPAPIEKTISKAKGQPREPQVYTLPPSREEMTKNQVSLTCLVKGFYPSDIAVEWESNGQPENNYKTTPPVLDSDGSFFLYSKLTVDKSRWQQGNVFSCSVMHEALHNHYTQKSLSLSPGGGGGGGGGGPATLCGAELVDALQFVCGDRGFYFNKPTGYGSSSRRAPQTGIVDECCARSCDLRRLEMYCAPLKPTKST

SEQ ID NO: 33 - protein, 306 aa, synthetic construct
DKTHTCPPCPAPELLGGPSVFLFPPKPKDTLMISRTPEVTCVVVDVSHEDPEVKFNWYVDGVEVHNAKTKPREEQYASTYRVVSVLTVLHQDWLNGKEYKCKVSNKALPAPIEKTISKAKGQPREPQVYTLPPSREEMTKNQVSLTCLVKGFYPSDIAVEWESNGQPENNYKTTPPVLDSDGSFFLYSKLTVDKSRWQQGNVFSCSVMHEALHNHYTQKSLSLSPGPAPAPAPAPAGPATLCGAELVDALQFVCGDRGFYFNKPTGYGSSSRRAPQTGIVDECCARSCDLRRLEMYCAPLKPTKST

SEQ ID NO: 34 - protein, 296 aa, synthetic construct
DKTHTCPPCPAPELLGGPSVFLFPPKPKDTLMISRTPEVTCVVVDVSHEDPEVKFNWYVDGVEVHNAKTKPREEQYASTYRVVSVLTVLHQDWLNGKEYKCKVSNKALPAPIEKTISKAKGQPREPQVYTLPPSREEMTKNQVSLTCLVKGFYPSDIAVEWESNGQPENNYKTTPPVLDSDGSFFLYSKLTVDKSRWQQGNVFSCSVMHEALHNHYTQKSLSLSPGGPATLCGAELVDALQFVCGDRGFYFNKPTGYGSSSRRAPQTGIVDECCARSCDLRRLEMYCAPLKPTKST

SEQ ID NO: 35 - protein, 346 aa, synthetic construct
HGEGTFTSDVSSYLEEQAAKEFIAWLVKGGGGSAPAPGGGGSDKTHTCPPCPAPELLGGPSVFLFPPKPKDTLMISRTPEVTCVVVDVSHEDPEVKFNWYVDGVEVHNAKTKPREEQYASTYRVVSVLTVYHMDWLNGKEYKCKVSNKALPAPIEKTISKAKGQPREPQVYTLPPSREEMTKNQVSLTCLVKGFYPSDIAVEWESNGQPENNYKTTPPVLDSDGSFFLYSKLTVDKSRWQQGNVFSCSVLHEALHNHYTQKSLSLSPGGGGGGGGGGPATLCGAELVDALQFVCGDRGFYFNKPTGYGSSSRRAPQTGIVDECCARSCDLRRLEMYCAPLKPTKST

SEQ ID NO: 36 - protein, 346 aa, synthetic construct
HGEGTFTSDVSSYLEEQAAKEFIAWLVKGGGGSAPAPGGGGSDKTHTCPPCPAPELLGGPSVFLFPPKPKDTLMISRTPEVTCVVVDVSHEDPEVKFNWYVDGVEVHNAKTKPREEQYASTYRVVSVLTVEHMDWLNGKEYKCKVSNKALPAPIEKTISKAKGQPREPQVYTLPPSREEMTKNQVSLTCLVKGFYPSDIAVEWESNGQPENNYKTTPPVLDSDGSFFLYSKLTVDKSRWQQGNVFSCSVLHEALHNHYTQKSLSLSPGGGGGGGGGGPATLCGAELVDALQFVCGDRGFYFNKPTGYGSSSRRAPQTGIVDECCARSCDLRRLEMYCAPLKPTKST

SEQ ID NO: 37 - protein, 346 aa, synthetic construct
HGEGTFTSDVSSYLEEQAAKEFIAWLVKGGGGSAPAPGGGGSDKTHTCPPCPAPELLGGPSVFLFPPKPKDTLMISRTPEVTCVVVDVSHEDPEVKFNWYVDGVEVHNAKTKPREEQYASTYRVVSVLTVEHWDWLNGKEYKCKVSNKALPAPIEKTISKAKGQPREPQVYTLPPSREEMTKNQVSLTCLVKGFYPSDIAVEWESNGQPENNYKTTPPVLDSDGSFFLYSKLTVDKSRWQQGNVFSCSVLHEALHNHYTQKSLSLSPGGGGGGGGGGPATLCGAELVDALQFVCGDRGFYFNKPTGYGSSSRRAPQTGIVDECCARSCDLRRLEMYCAPLKPTKST

SEQ ID NO: 38 - protein, 11 aa, synthetic construct
GSAPAPGGGGS

SEQ ID NO: 39 - protein, 24 aa, synthetic construct
GGGGSGGGGSGGGGSGGGGSGAHS

SEQ ID NO: 40 - protein, 16 aa, synthetic construct
ASGAGSTTLEVLFQGP

SEQ ID NO: 41 - protein, 8 aa, synthetic construct
GGGGGGGG

SEQ ID NO: 42 - protein, 10 aa, synthetic construct
PAPAPAPAPA